European Patent Application EP 4 335 511 A2, published March 13, 2024. Title: SMALL MOLECULE TRAIL GENE INDUCTION BY NORMAL AND TUMOR CELLS AS AN ANTICANCER THERAPY. Applicant: The Penn State Research Foundation. Application EP. The sequence listing filed with the application follows.

SEQUENCE LISTING (4 sequences)

SEQ ID NO: 1 - DNA, 21 bp, synthetic construct
  misc_feature 1..21: note = Forward primer for TRAIL
  source 1..21: mol_type = other DNA
cagaggaagaagcaacacatt

SEQ ID NO: 2 - DNA, 28 bp, synthetic construct
  misc_feature 1..28: note = Reverse primer for TRAIL
  source 1..28: mol_type = other DNA
ggttgatgattcccaggagtttattttg

SEQ ID NO: 3 - DNA, 20 bp, synthetic construct
  misc_feature 1..20: note = Forward primer for GAPDH
  source 1..20: mol_type = other DNA
ccacatcgctcagacaccat

SEQ ID NO: 4 - DNA, 26 bp, synthetic construct
  misc_feature 1..26: note = Reverse primer for GAPDH
  source 1..26: mol_type = other DNA
ggcaacaatatccactttaccagagt